European Patent Application EP 4 491 736 A1, published January 15, 2025. Title: A microorganism culture medium composition for retinol production comprising antioxidant. Applicant: 씨제이제일제당 주식회사. Application KR. The sequence listing filed with the application follows.

SEQUENCE LISTING (70 sequences)

SEQ ID NO: 1 - DNA, 2022 bp, Xanthophyllomyces dendrorhous
  source 1..2022: mol_type = genomic DNA
atgacggctctcgcatattaccagatccatctgatctatactctcccaattcttggtcttctcggcctgctcacttccccgattttgacaaaatttgacatctacaaaatatcgatcctcgtatttattgcgtttagtgcaaccacaccatgggactcatggatcatcagaaatggcgcatggacatatccatcagcggagagtggccaaggcgtgtttggaacgtttctagatgttccatatgaagagtacgctttctttgtcattcaaaccgtaatcaccggcttggtctacgtcttggcaactaggcaccttctcccatctctcgcgcttcccaagactagatcgtccgccctttctctcgcgctcaaggcgctcatccctctgcccattatctacctatttaccgctcaccccagcccatcgcccgacccgctcgtgacagatcactacttctacatgcgggcactctccttactcatcaccccacctaccatgctcttggcagcattatcaggcgaatatgctttcgattggaaaagtggccgagcaaagtcaactattgcagcaatcatgatcccgacggtgtatctgatttgggtagattatgttgctgtcggtcaagactcttggtcgatcaacgatgagaagattgtagggtggaggcttggaggtgtactacccattgaggaagctatgttcttcttactgacgaatctaatgattgttctgggtctgtctgcctgcgatcatactcaggccctatacctgctacacggtcgaactatttatggcaacaaaaagatgccatcttcatttcccctcattacaccgcctgtgctctccctgttttttagcagccgaccatactcttctcagccaaaacgtgacttggaactggcagtcaagttgttggaggaaaagagccggagcttttttgttgcctcggctggatttcctagcgaagttagggagaggctggttggactatacgcattctgccgggtgactgatgatcttatcgactctcctgaagtatcttccaacccgcatgccacaattgacatggtctccgattttcttaccctactatttgggcccccgctacacccttcgcaacctgacaagatcctttcttcgcctttacttcctccttcgcacccttcccgacccacgggaatgtatcccctcccgcctcctccttcgctctcgcctgccgagctcgttcaattccttaccgaaagggttcccgttcaataccatttcgccttcaggttgctcgctaagttgcaagggctgatccctcgatacccactcgacgaactccttagaggatacaccactgatcttatctttcccttatcgacagaggcagtccaggctcggaagacgcctatcgagaccacagctgacttgctggactatggtctatgtgtagcaggctcagtcgccgagctattggtctatgtctcttgggcaagtgcaccaagtcaggtccctgccaccatagaagaaagagaagctgtgttagtggcaagccgagagatgggaactgcccttcagttggtgaacattgctagggacattaaaggggacgcaacagaagggagattttacctaccactctcattctttggtcttcgggatgaatcaaagcttgcgatcccgactgattggacggaacctcggcctcaagatttcgacaaactcctcagtctatctccttcgtccacattaccatcttcaaacgcctcagaaagcttccggttcgaatggaagacgtactcgcttccattagtcgcctacgcagaggatcttgccaaacattcttataagggaattgaccgacttcctaccgaggttcaagcgggaatgcgagcggcttgcgcgagctacctactgatcggccgagagatcaaagtcgtttggaaaggagacgtcggagagagaaggacagttgccggatggaggagagtacggaaagtcttgagtgtggtcatgagcggatgggaagggcagtaa

SEQ ID NO: 2 - DNA, 1749 bp, Xanthophyllomyces dendrorhous
  source 1..1749: mol_type = genomic DNA
atgggaaaagaacaagatcaggataaacccacagctatcatcgtgggatgtggtatcggtggaatcgccactgccgctcgtcttgctaaagaaggtttccaggtcacggtgttcgagaagaacgactactccggaggtcgatgctctttaatcgagcgagatggttatcgattcgatcaggggcccagtttgctgctcttgccagatctcttcaagcagacattcgaagatttgggagagaagatggaagattgggtcgatctcatcaagtgtgaacccaactatgtttgccacttccacgatgaagagactttcactctttcaaccgacatggcgttgctcaagcgggaagtcgagcgttttgaaggcaaagatggatttgatcggttcttgtcgtttatccaagaagcccacagacattacgagcttgctgtcgttcacgtcctgcagaagaacttccctggcttcgcagcattcttacggctacagttcattggccaaatcctggctcttcaccccttcgagtctatctggacaagagtttgtcgatatttcaagaccgacagattacgaagagtcttctcgtttgcagtgatgtacatgggtcaaagcccatacagtgcgcccggaacatattccttgctccaatacaccgaattgaccgagggcatctggtatccgagaggaggcttttggcaggttcctaatactcttcttcagatcgtcaagcgcaacaatccctcagccaagttcaatttcaacgctccagtttcccaggttcttctctctcctgccaaggaccgagcgactggtgttcgacttgaatccggcgaggaacatcacgccgatgttgtgattgtcaatgctgacctcgtttacgcctccgagcacttgattcctgacgatgccagaaacaagattggccaactgggtgaagtcaagagaagttggtgggctgacttagttggtggaaagaagctcaagggaagttgcagtagtttgagcttctactggagcatggaccgaatcgtggacggtctgggcggacacaatatcttcttggccgaggacttcaagggatcattcgacacaatcttcgaggagttgggtctcccagccgatccttccttttacgtgaacgttccctcgcgaatcgatccttctgccgctcccgaaggcaaagatgctatcgtcattcttgtgccgtgtggccatatcgacgcttcgaaccctcaagattacaacaagcttgttgctcgggcaaggaagtttgtgatccacacgctttccgccaagcttggacttcccgactttgaaaaaatgattgtggcagagaaggttcacgatgctccctcttgggagaaagaattcaacctcaaggacggaagcatcttgggactggctcacaactttatgcaagttcttggtttcaggccgagcaccagacatcccaagtatgacaagttgttctttgtcggggcttcgactcatcccggaactggggttcccatcgtcttggctggagccaagttaactgccaaccaagttctcgaatcctttgaccgatccccagctccagatcccaatatgtcactctccgtaccatatggaaaacctctcaaatcaaatggaacgggtatcgattctcaggtccagctgaagttcatggatttggagagatgggtataccttttggtgttgttgattggggccgtgatcgctcgatccgttggtgttcttgctttctga

SEQ ID NO: 3 - DNA, 2804 bp, synthetic construct
  source 1..2804: mol_type = other DNA
agagaccgggttggcggcgcatttgtgtcccaaaaaacagccccaattgccccaattgaccccaaattgacccagtagcgggcccaaccccggcgagagcccccttctccccacatatcaaacctcccccggttcccacacttgccgttaagggcgtagggtactgcagtctggaatctacgcttgttcagactttgtactagtttctttgtctggccatccgggtaacccatgccggacgcaaaatagactactgaaaatttttttgctttgtggttgggactttagccaagggtataaaagaccaccgtccccgaattacctttcctcttcttttctctctctccttgtcaactcacacccgaaatcgttaagcatttccttctgagtataagaatcattcaaaatggtgagtttcagaggcagcagcaattgccacgggctttgagcacacggccgggtgtggtcccattcccatcgacacaagacgccacgtcatccgaccagcactttttgcagtactaaccgcagacggctctcgcatattaccagatccatctgatctatactctcccaattcttggtcttctcggtctgctcacttccccgattttgacaaaatttgacatctacaaaatatcgatcctcgtatttattgcgtttagtgcaaccacaccatgggactcatggatcatcagaaatggcgcatggacatatccatcagcggagagtggccaaggcgtgtttggaacgtttctagatgttccatatgaagagtacgctttctttgtcattcaaaccgtaatcaccggcttggtctacgtcttggcaactaggcaccttctcccatctctcgcgcttcccaagactagatcgtccgccctttctctcgcgctcaaggcgctcatccctctgcccattatctacctatttaccgctcaccccagcccatcgcccgacccgctcgtgacagatcactacttctacatgcgggcactctccttactcatcaccccacctaccatgctcttggcagcattatcaggcgaatatgctttcgattggaaaagtggccgagcaaagtcaactattgcagcaatcatgatcccgacggtgtatctgatttgggtagattatgttgctgtcggtcaagactcttggtcgatcaacgatgagaagattgtagggtggaggcttggaggtgtactacccattgaggaagctatgttcttcttactgacgaatctaatgattgttctgggtctgtctgcctgcgatcatactcaggccctatacctgctacacggtcgaactatttatggcaacaaaaagatgccatcttcatttcccctcattacaccgcctgtgctctccctgttttttagcagccgaccatactcttctcagccaaaacgtgacttggaactggcagtcaagttgttggaggaaaagagccggagcttttttgttgcctcggctggatttcctagcgaagttagggagaggctggttggactatacgcattctgccgggtgactgatgatcttatcgactctcctgaagtatcttccaacccgcatgccacaattgacatggtctccgattttcttaccctactatttgggcccccgctacacccttcgcaacctgacaagatcctttcttcgcctttacttcctccttcgcacccttcccgacccacgggaatgtatcccctcccgcctcctccttcgctctcgcctgccgagctcgttcaattccttaccgaaagggttcccgttcaataccatttcgccttcaggttgctcgctaagttgcaagggctgatccctcgatacccactcgacgaactccttagaggatacaccactgatcttatctttcctttatcgacagaggcagtccaggctcggaagacgcctatcgagaccacagctgacttgctggactatggtctatgtgtagcaggctcagtcgccgagctattggtctatgtctcttgggcaagtgcaccaagtcaggtccctgccaccatagaagaaagagaagctgtgttagtggcaagccgagagatgggaactgcccttcagttggtgaacattgctagggacattaaaggggacgcaacagaagggagattttacctaccactctcattctttggtcttcgggatgaatcaaagcttgcgatcccgactgattggacggaacctcggcctcaagatttcgacaaactcctcagtctatctccttcgtccacattaccatcttcaaacgcctcagaaagcttccggttcgaatggaagacgtactcgcttccattagtcgcctacgcagaggatcttgccaaacattcttataagggaattgaccgacttcctaccgaggttcaagcgggaatgcgagcggcttgcgcgagctacctactgatcggccgagagatcaaagtcgtttggaaaggagacgtcggagagagaaggacagttgccggatggaggagagtacggaaagtcttgagtgtggtcatgagcggatgggaagggcagtaactcgagtcatgtaattagttatgtcacgcttacattcacgccctccccccacatccgctctaaccgaaaaggaaggagttagacaacctgaagtctaggtccctatttatttttttatagttatgttagtattaagaacgttatttatatttcaaatttttcttttttttctgtacagacgcgtgtacgcatgtaacattatactgaaaaccttgcttgagaaggttttgggacgctcgaaggctttaatttgc

SEQ ID NO: 4 - DNA, 2531 bp, synthetic construct
  source 1..2531: mol_type = other DNA
agagaccgggttggcggcgcatttgtgtcccaaaaaacagccccaattgccccaattgaccccaaattgacccagtagcgggcccaaccccggcgagagcccccttctccccacatatcaaacctcccccggttcccacacttgccgttaagggcgtagggtactgcagtctggaatctacgcttgttcagactttgtactagtttctttgtctggccatccgggtaacccatgccggacgcaaaatagactactgaaaatttttttgctttgtggttgggactttagccaagggtataaaagaccaccgtccccgaattacctttcctcttcttttctctctctccttgtcaactcacacccgaaatcgttaagcatttccttctgagtataagaatcattcaaaatggtgagtttcagaggcagcagcaattgccacgggctttgagcacacggccgggtgtggtcccattcccatcgacacaagacgccacgtcatccgaccagcactttttgcagtactaaccgcagggaaaagaacaagatcaggataaacccacagctatcatcgtgggatgtggtatcggtggaatcgccactgccgctcgtcttgctaaagaaggtttccaggtcacggtgttcgagaagaacgactactccggaggtcgatgctctttaatcgagcgagatggttatcgattcgatcaggggcccagtttgctgctcttgccagatctcttcaagcagacattcgaagatttgggagagaagatggaagattgggtcgatctcatcaagtgtgaacccaactatgtttgccacttccacgatgaagagactttcactctttcaaccgacatggcgttgctcaagcgggaagtcgagcgttttgaaggcaaagatggatttgatcggttcttgtcgtttatccaagaagcccacagacattacgagcttgctgtcgttcacgtcctgcagaagaacttccctggcttcgcagcattcttacggctacagttcattggccaaatcctggctcttcaccccttcgagtctatctggacaagagtttgtcgatatttcaagaccgacagattacgaagagtcttctcgtttgcagtgatgtacatgggtcaaagcccatacagtgcgcccggaacatattccttgctccaatacaccgaattgaccgagggcatctggtatccgagaggaggcttttggcaggttcctaatactcttcttcagatcgtcaagcgcaacaatccctcagccaagttcaatttcaacgctccagtttcccaggttcttctctctcctgccaaggaccgagcgactggtgttcgacttgaatccggcgaggaacatcacgccgatgttgtgattgtcaatgctgacctcgtttacgcctccgagcacttgattcctgacgatgccagaaacaagattggccaactgggtgaagtcaagagaagttggtgggctgacttagttggtggaaagaagctcaagggaagttgcagtagtttgagcttctactggagcatggaccgaatcgtggacggtctgggcggacacaatatcttcttggccgaggacttcaagggatcattcgacacaatcttcgaggagttgggtctcccagccgatccttccttttacgtgaacgttccctcgcgaatcgatccttctgccgctcccgaaggcaaagatgctatcgtcattcttgtgccgtgtggccatatcgacgcttcgaaccctcaagattacaacaagcttgttgctcgggcaaggaagtttgtgatccacacgctttccgccaagcttggacttcccgactttgaaaaaatgattgtggcagagaaggttcacgatgctccctcttgggagaaagaattcaacctcaaggacggaagcatcttgggactggctcacaactttatgcaagttcttggtttcaggccgagcaccagacatcccaagtatgacaagttgttctttgtcggggcttcgactcatcccggaactggggttcccatcgtcttggctggagccaagttaactgccaaccaagttctcgaatcctttgaccgatccccagctccagatcccaatatgtcactctccgtaccatatggaaaacctctcaaatcaaatggaacgggtatcgattctcaggtccagctgaagttcatggatttggagagatgggtataccttttggtattgttgattggggccgtgatcgctcgatccgttggtgttcttgctttctgactcgagtcatgtaattagttatgtcacgcttacattcacgccctccccccacatccgctctaaccgaaaaggaaggagttagacaacctgaagtctaggtccctatttatttttttatagttatgttagtattaagaacgttatttatatttcaaatttttcttttttttctgtacagacgcgtgtacgcatgtaacattatactgaaaaccttgcttgagaaggttttgggacgctcgaaggctttaatttgc

SEQ ID NO: 5 - DNA, 1533 bp, Yarrowia lipolytica
  source 1..1533: mol_type = genomic DNA
tgcctcctgtctgactcgtcattgccgcctttggagtacgactccaactatgagtgtgcttggatcactttgacgatacattcttcgttggaggctgtgggtctgacagctgcgttttcggcgcggttggccgacaacaatatcagctgcaacgtcattgctggctttcatcatgatcacatttttgtcggcaaaggcgacgcccagagagccattgacgttctttctaatttggaccgatagccgtatagtccagtctatctataagttcaactaactcgtaactattaccataacatatacttcactgccccagataaggttccgataaaaagttctgcagactaaatttatttcagtctcctcttcaccaccaaaatgccctcctacgaagctcgagctaacgtccacaagtccgcctttgccgctcgagtgctcaagctcgtggcagccaagaaaaccaacctgtgtgcttctctggatgttaccaccaccaaggagctcattgagcttgccgataaggtcggaccttatgtgtgcatgatcaagacccatatcgacatcattgacgacttcacctacgccggcactgtgctccccctcaaggaacttgctcttaagcacggtttcttcctgttcgaggacagaaagttcgcagatattggcaacactgtcaagcaccagtacaagaacggtgtctaccgaatcgccgagtggtccgatatcaccaacgcccacggtgtacccggaaccggaatcattgctggcctgcgagctggtgccgaggaaactgtctctgaacagaagaaggaggacgtctctgactacgagaactcccagtacaaggagttcctggtcccctctcccaacgagaagctggccagaggtctgctcatgctggccgagctgtcttgcaagggctctctggccactggcgagtactccaagcagaccattgagcttgcccgatccgaccccgagtttgtggttggcttcattgcccagaaccgacctaagggcgactctgaggactggcttattctgacccccggggtgggtcttgacgacaagggagacgctctcggacagcagtaccgaactgttgaggatgtcatgtctaccggaacggatatcataattgtcggccgaggtctgtacggccagaaccgagatcctattgaggaggccaagcgataccagaaggctggctgggaggcttaccagaagattaactgttagaggttagactatggatatgtcatttaactgtgtatatagagagcgtgcaagtatggagcgcttgttcagcttgtatgatggtcagacgacctgtctgatcgagtatgtatgatactgcacaacctgtgtatccgcatgatctgtccaatggggcatgttgttgtgtttctcgatacggagatgctgggtacaagtagctaatacgattgaactacttatacttatatgaggcttgaagaaagctgacttgtgtatgacttattctcaactacatccccagtcacaataccacca

SEQ ID NO: 6 - DNA, 30 bp, synthetic construct
  source 1..30: mol_type = other DNA
gtgcgcttctctcgtctcggtaaccctgtc

SEQ ID NO: 7 - DNA, 44 bp, synthetic construct
  source 1..44: mol_type = other DNA
atgcgccgccaacccggtctctggggtgtggtggatggggtgtg

SEQ ID NO: 8 - DNA, 44 bp, synthetic construct
  source 1..44: mol_type = other DNA
cacaccccatccaccacaccccagagaccgggttggcggcgcat

SEQ ID NO: 9 - DNA, 39 bp, synthetic construct
  source 1..39: mol_type = other DNA
cgccgccaacccggtctcttgaagacgaaagggcctccg

SEQ ID NO: 10 - DNA, 39 bp, synthetic construct
  source 1..39: mol_type = other DNA
cggaggccctttcgtcttcaagagaccgggttggcggcg

SEQ ID NO: 11 - DNA, 40 bp, synthetic construct
  source 1..40: mol_type = other DNA
gacgagtcagacaggaggcatcagacagatactcgtcgcg

SEQ ID NO: 12 - DNA, 40 bp, synthetic construct
  source 1..40: mol_type = other DNA
cgcgacgagtatctgtctgatgcctcctgtctgactcgtc

SEQ ID NO: 13 - DNA, 44 bp, synthetic construct
  source 1..44: mol_type = other DNA
atgacgagtcagacaggaggcatggtggtattgtgactggggat

SEQ ID NO: 14 - DNA, 44 bp, synthetic construct
  source 1..44: mol_type = other DNA
atccccagtcacaataccaccatgcctcctgtctgactcgtcat

SEQ ID NO: 15 - DNA, 44 bp, synthetic construct
  source 1..44: mol_type = other DNA
cggcgtccttctcgtagtccgcttttggtggtgaagaggagact

SEQ ID NO: 16 - DNA, 44 bp, synthetic construct
  source 1..44: mol_type = other DNA
agtctcctcttcaccaccaaaagcggactacgagaaggacgccg

SEQ ID NO: 17 - DNA, 30 bp, synthetic construct
  source 1..30: mol_type = other DNA
ccactcgtcaccaacagtgccgtgtgttgc

SEQ ID NO: 18 - DNA, 24 bp, synthetic construct
  source 1..24: mol_type = other DNA
tcgtacgtctataccaacagatgg

SEQ ID NO: 19 - DNA, 24 bp, synthetic construct
  source 1..24: mol_type = other DNA
cgcatacacacacactgccggggg

SEQ ID NO: 20 - DNA, 550 bp, Yarrowia lipolytica
  source 1..550: mol_type = genomic DNA
tccacacgtcgttcttttttccttagccttttttgcagtgcgcgtgtcccaaaccccagctctacacaccagcacaaacaaagttaagctcagggttgtcgttgaggtcgcttactgtagtcagtgctcgtatggttcgttcaattttcgccaaaaatcgttttgcctttgtatcttgggaataacatcaactgtggttcttcaacaggcctaaggaacgaaacaagccggaccaagatcaggttcaaggtgagtactgagaaggaatagaaggcctaaaggcgcaaaccgacaggtggcaacagctccacaccgaccacgaaggccacgaaatcaaggggtcctaaagttagtctttgtggcctcgacggtcagcgaaaacgcgagaccacaacgcgatcagaaccaggacctaaacaacacaggacggggtcacaataggcttgaacagcaagtacaagctgtgatctctctatatttgattctcaaaccacccctgactacttcagcgcctctgtgacacagcccccctatcatccgactaacacag

SEQ ID NO: 21 - DNA, 31 bp, synthetic construct
  source 1..31: mol_type = other DNA
gacaatgcctcgaggaggtttaaaagtaact

SEQ ID NO: 22 - DNA, 41 bp, synthetic construct
  source 1..41: mol_type = other DNA
gcgccgccaacccggtctctctgtgttagtcggatgatagg

SEQ ID NO: 23 - DNA, 41 bp, synthetic construct
  source 1..41: mol_type = other DNA
cctatcatccgactaacacagagagaccgggttggcggcgc

SEQ ID NO: 24 - DNA, 42 bp, synthetic construct
  source 1..42: mol_type = other DNA
gacgagtcagacaggaggcactgcggttagtactgcaaaaag

SEQ ID NO: 25 - DNA, 42 bp, synthetic construct
  source 1..42: mol_type = other DNA
ctttttgcagtactaaccgcagtgcctcctgtctgactcgtc

SEQ ID NO: 26 - DNA, 44 bp, synthetic construct
  source 1..44: mol_type = other DNA
atgcgccgccaacccggtctcttggtggtattgtgactggggat

SEQ ID NO: 27 - DNA, 44 bp, synthetic construct
  source 1..44: mol_type = other DNA
atccccagtcacaataccaccaagagaccgggttggcggcgcat

SEQ ID NO: 28 - DNA, 41 bp, synthetic construct
  source 1..41: mol_type = other DNA
ctttccaatagctgcttgtagctgcggttagtactgcaaaa

SEQ ID NO: 29 - DNA, 41 bp, synthetic construct
  source 1..41: mol_type = other DNA
ttttgcagtactaaccgcagctacaagcagctattggaaag

SEQ ID NO: 30 - DNA, 30 bp, synthetic construct
  source 1..30: mol_type = other DNA
gcttaatgtgattgatctcaaacttgatag

SEQ ID NO: 31 - DNA, 24 bp, synthetic construct
  source 1..24: mol_type = other DNA
gctgtctctgcgagagcacgtcga

SEQ ID NO: 32 - DNA, 24 bp, synthetic construct
  source 1..24: mol_type = other DNA
ggttcgcacaacttctcgggtggc

SEQ ID NO: 33 - DNA, 1017 bp, Haematococcus pluvialis
  source 1..1017: mol_type = genomic DNA
atgatccgagcgatgcacaaccgggcgcccacacctcgaactcgagtgtctcatccacgctcacatagggctctggcacatgtctcagccgtagcaacagcagggcaggtggcagaggtccactctgctcctgcctttgacttcgagatgtacatgagagacagagctgagatggtcaacaaggctcttgatgctgcattgccatctagataccctgaggtgctggttgattccatgaggtactccgtacttgcgggtggcaagcgcgtgaggcctgccctgacactggctgcgtgcgaccttgtaggaggggacatggccactgccctacccaccgcatgtgccatggagatgatccacaccatgagcctcatccatgatgacctgccagccatggacaatgacgacttcaggcgaggtcggcccacaaaccataaggtgtatggtgaggacattgccatccttgctggtgacgcgctgctgtcctttgcctttgagcacatcgcccgggacaccaaaggcgtgccggctgatgcggtgctgaaggtcatcatggagctgggccgggccgtgggcgcgcagggcctatcagcaggccaggctgttgacataaagagcgagggccaggaggtggggctggaggtgctggagtacatccaccaccacaagacagctgcactgctggaggcggcagtggtgtgcggcgcactggtgggcggggccgacaccgccaccgtggagaagctgcgcaagtacgcgctgaacattgggctggccttccaggtgattgatgacatcctggacgtcactcaaaccaccgaaaccttgggcaagaccgcagccaaagacctggcggtgaacaagaccacctatcccaagctgctgggtctggaagccagcaggaaggtggcggacgacttgatcagggaggctatagcacagttagacgagtttgagcctgcacgcaaggcgcccatggtggccctggcccacctcatagggtaccgcaagaactga

SEQ ID NO: 34 - DNA, 1793 bp, synthetic construct
  source 1..1793: mol_type = other DNA
agagaccgggttggcggcgcatttgtgtcccaaaaaacagccccaattgccccaattgaccccaaattgacccagtagcgggcccaaccccggcgagagcccccttctccccacatatcaaacctcccccggttcccacacttgccgttaagggcgtagggtactgcagtctggaatctacgcttgttcagactttgtactagtttctttgtctggccatccgggtaacccatgccggacgcaaaatagactactgaaaatttttttgctttgtggttgggactttagccaagggtataaaagaccaccgtccccgaattacctttcctcttcttttctctctctccttgtcaactcacacccgaaatcgttaagcatttccttctgagtataagaatcattcaaaatggtgagtttcagaggcagcagcaattgccacgggctttgagcacacggccgggtgtggtcccattcccatcgacacaagacgccacgtcatccgaccagcactttttgcagtactaaccgcagatccgagccatgcacaaccgagcccccaccccccgaacccgagtgtctcacccccgatctcaccgagccctggcccacgtgtctgccgtggccaccgccggccaggtggccgaggtgcactctgcccccgccttcgacttcgagatgtacatgcgagaccgagccgagatggtgaacaaggccctggacgccgccctgccctctcgataccccgaggtgctggtggactctatgcgatactctgtgctggccggcggcaagcgagtgcgacccgccctgaccctggccgcctgtgacctggtgggcggcgacatggccaccgccctgcccaccgcctgtgccatggagatgatccacaccatgtctctgatccacgacgacctgcccgccatggacaacgacgacttccgacgaggccgacccaccaaccacaaggtgtacggcgaggacatcgccatcctggccggcgacgccctgctgtctttcgccttcgagcacatcgcccgagacaccaagggcgtgcccgccgacgccgtgctgaaggtgatcatggagctgggccgagccgtgggcgcccagggcctgtctgccggccaggccgtggacatcaagtctgagggccaggaggtgggcctggaggtgctggagtacatccaccaccacaagaccgccgccctgctggaggccgccgtggtgtgtggcgccctggtgggcggcgccgacaccgccaccgtggagaagctgcgaaagtacgccctgaacatcggcctggccttccaggtgatcgacgacatcctggacgtgacccagaccaccgagaccctgggcaagaccgccgccaaggacctggccgtgaacaagaccacctaccccaagctgctgggcctggaggcctctcgaaaggtggccgacgacctgatccgagaggccatcgcccagctggacgagttcgagcccgcccgaaaggcccccatggtggccctggcccacctgatcggctaccgaaagaactagtcatgtaattagttatgtcacgcttacattcacgccctccctccacatccgctctaaccgaaaaggaaggagttagacaacctgaagtctaggtccctatttatttttttatagttatgttagtattaagaacgttatttatatttcaaatttttcttttttttctgtacagacgcgtgtacgcatgtaacattatactgaaaaccttgcttgagaaggttttgggacgctcgaaggctttaatttgc

SEQ ID NO: 35 - DNA, 30 bp, synthetic construct
  source 1..30: mol_type = other DNA
aagacaaggcttcggaagcgagaaccgcaa

SEQ ID NO: 36 - DNA, 44 bp, synthetic construct
  source 1..44: mol_type = other DNA
atgcgccgccaacccggtctctgtgtttggcggtgtgagttgtc

SEQ ID NO: 37 - DNA, 44 bp, synthetic construct
  source 1..44: mol_type = other DNA
gacaactcacaccgccaaacacagagaccgggttggcggcgcat

SEQ ID NO: 38 - DNA, 44 bp, synthetic construct
  source 1..44: mol_type = other DNA
atgacgagtcagacaggaggcactgcggttagtactgcaaaaag

SEQ ID NO: 39 - DNA, 44 bp, synthetic construct
  source 1..44: mol_type = other DNA
ctttttgcagtactaaccgcagtgcctcctgtctgactcgtcat

SEQ ID NO: 40 - DNA, 44 bp, synthetic construct; identical to SEQ ID NO: 26
  source 1..44: mol_type = other DNA

SEQ ID NO: 41 - DNA, 44 bp, synthetic construct; identical to SEQ ID NO: 27
  source 1..44: mol_type = other DNA

SEQ ID NO: 42 - DNA, 44 bp, synthetic construct
  source 1..44: mol_type = other DNA
atatggagtgttatttgaaggggcaaattaaagccttcgagcgt

SEQ ID NO: 43 - DNA, 44 bp, synthetic construct
  source 1..44: mol_type = other DNA
acgctcgaaggctttaatttgccccttcaaataacactccatat

SEQ ID NO: 44 - DNA, 30 bp, synthetic construct
  source 1..30: mol_type = other DNA
gtgtccaagtacgaacgccaatgcaagatt

SEQ ID NO: 45 - DNA, 24 bp, synthetic construct
  source 1..24: mol_type = other DNA
ccagttatttgtaccatgcggtgg

SEQ ID NO: 46 - DNA, 24 bp, synthetic construct
  source 1..24: mol_type = other DNA
ccatcttgtgtcgcgacgacgaaa

SEQ ID NO: 47 - DNA, 44 bp, synthetic construct
  source 1..44: mol_type = other DNA
cccacctcctcctcctgctcccccggcagcccctgccgcccctg

SEQ ID NO: 48 - DNA, 44 bp, synthetic construct
  source 1..44: mol_type = other DNA
atgacgagtcagacaggaggcacctagttagtcagaatttttgt

SEQ ID NO: 49 - DNA, 44 bp, synthetic construct
  source 1..44: mol_type = other DNA
acaaaaattctgactaactaggtgcctcctgtctgactcgtcat

SEQ ID NO: 50 - DNA, 44 bp, synthetic construct
  source 1..44: mol_type = other DNA
taccggtcggtagctacaatactggtggtattgtgactggggat

SEQ ID NO: 51 - DNA, 44 bp, synthetic construct
  source 1..44: mol_type = other DNA
atccccagtcacaataccaccagtattgtagctaccgaccggta

SEQ ID NO: 52 - DNA, 44 bp, synthetic construct
  source 1..44: mol_type = other DNA
cgtgtagatccaccacatacaccctagttagtcagaatttttgt

SEQ ID NO: 53 - DNA, 44 bp, synthetic construct
  source 1..44: mol_type = other DNA
acaaaaattctgactaactagggtgtatgtggtggatctacacg

SEQ ID NO: 54 - DNA, 44 bp, synthetic construct
  source 1..44: mol_type = other DNA
aagtaggaaacatgatggcctcttcttcctcttttgtaatgtac

SEQ ID NO: 55 - DNA, 24 bp, synthetic construct
  source 1..24: mol_type = other DNA
cccaactctcgaggaaatggccat

SEQ ID NO: 56 - DNA, 24 bp, synthetic construct
  source 1..24: mol_type = other DNA
ctggggatcttttccatccttgtt

SEQ ID NO: 57 - protein, 275 aa, Uncultured marine bacterium 66A03 [sequence omitted]

SEQ ID NO: 58 - DNA, 1604 bp, synthetic construct
  source 1..1604: mol_type = other DNA
agagaccgggttggcggcgcatttgtgtcccaaaaaacagccccaattgccccaattgaccccaaattgacccagtagcgggcccaaccccggcgagagcccccttctccccacatatcaaacctcccccggttcccacacttgccgttaagggcgtagggtactgcagtctggaatctacgcttgttcagactttgtactagtttctttgtctggccatccgggtaacccatgccggacgcaaaatagactactgaaaatttttttgctttgtggttgggactttagccaagggtataaaagaccaccgtccccgaattacctttcctcttcttttctctctctccttgtcaactcacacccgaaatcgttaagcatttccttctgagtataagaatcattcaaaatggtgagtttcagaggcagcagcaattgccacgggctttgagcacacggccgggtgtggtcccattcccatcgacacaagacgccacgtcatccgaccagcactttttgcagtactaaccgcagggcctgatgctgatcgactggtgtgccctggccctggtggtgttcatcggcctgccccacggcgccctggacgccgccatctctttctctatgatctcttctgccaagcgaatcgcccgactggccggcatcctgctgatctacctgctgctggccaccgccttcttcctgatctggtaccagctgcccgccttctctctgctgatcttcctgctgatctctatcatccacttcggcatggccgacttcaacgcctctccctctaagctgaagtggccccacatcatcgcccacggcggcgtggtgaccgtgtggctgcccctgatccagaagaacgaggtgaccaagctgttctctatcctgaccaacggccccacccccatcctgtgggacatcctgctgatcttcttcctgtgttggtctatcggcgtgtgtctgcacacctacgagaccctgcgatctaagcactacaacatcgccttcgagctgatcggcctgatcttcctggcctggtacgccccccccctggtgaccttcgccacctacttctgtttcatccactctcgacgacacttctctttcgtgtggaagcagctgcagcacatgtcttctaagaagatgatgatcggctctgccatcatcctgtcttgtacctcttggctgatcggcggcggcatctacttcttcctgaactctaagatgatcgcctctgaggccgccctgcagaccgtgttcatcggcctggccgccctgaccgtgccccacatgatcctgatcgacttcatcttccgaccccactcttctcgaatcaagatcaagaactagtcatgtaattagttatgtcacgcttacattcacgccctccctccacatccgctctaaccgaaaaggaaggagttagacaacctgaagtctaggtccctatttatttttttatagttatgttagtattaagaacgttatttatatttcaaatttttcttttttttctgtacagacgcgtgtacgcatgtaacattatactgaaaaccttgcttgagaaggttttgggacgctcgaaggctttaatttgc

SEQ ID NO: 59 - DNA, 45 bp, synthetic construct
  source 1..45: mol_type = other DNA
gtacccggggatcctctagaggcgtttcaggtggttgcgtgagtg

SEQ ID NO: 60 - DNA, 53 bp, synthetic construct
  source 1..53: mol_type = other DNA
gacacaaatgcgccgccaacccggtctctgcggcggttcgtggttcgtgtttc

SEQ ID NO: 61 - DNA, 53 bp, synthetic construct
  source 1..53: mol_type = other DNA
gaaacacgaaccacgaaccgccgcagagaccgggttggcggcgcatttgtgtc

SEQ ID NO: 62 - DNA, 49 bp, synthetic construct
  source 1..49: mol_type = other DNA
gacgagtcagacagatactcgtcggcaaattaaagccttcgagcgtccc

SEQ ID NO: 63 - DNA, 49 bp, synthetic construct
  source 1..49: mol_type = other DNA
gggacgctcgaaggctttaatttgccgacgagtatctgtctgactcgtc

SEQ ID NO: 64 - DNA, 50 bp, synthetic construct
  source 1..50: mol_type = other DNA
caggaagaagtagatgccgccgccgcaaaggcctgtttctcggtgtacag

SEQ ID NO: 65 - DNA, 50 bp, synthetic construct
  source 1..50: mol_type = other DNA
ctgtacaccgagaaacaggcctttgcggcggcggcatctacttcttcctg

SEQ ID NO: 66 - DNA, 48 bp, synthetic construct
  source 1..48: mol_type = other DNA
gcagcagtcatacatgttctgaggcaaattaaagccttcgagcgtccc

SEQ ID NO: 67 - DNA, 48 bp, synthetic construct
  source 1..48: mol_type = other DNA
gggacgctcgaaggctttaatttgcctcagaacatgtatgactgctgc

SEQ ID NO: 68 - DNA, 45 bp, synthetic construct
  source 1..45: mol_type = other DNA
gcctgcaggtcgactctagactactttgtgcagattgaggccaag

SEQ ID NO: 69 - DNA, 24 bp, synthetic construct
  source 1..24: mol_type = other DNA
cttgaccttgtagagctgaccggc

SEQ ID NO: 70 - DNA, 24 bp, synthetic construct
  source 1..24: mol_type = other DNA
cactactttcgccaccaagatggg